European Patent Application EP 4 219 470 A1, published August 2, 2023. Title: JAK1 SELECTIVE INHIBITORS. Applicant: ASTRAZENECA AB. Application EP, filed January 16, 2018. The sequence listing filed with the application follows.

SEQUENCE LISTING (2 sequences)

SEQ ID NO: 1 - protein, 16 aa, synthetic construct
  REGION 1..16: note = JAK kinases peptide substrates
KKHTDDGYMPMSPGVA

SEQ ID NO: 2 - protein, 14 aa, synthetic construct
  REGION 1..14: note = JAK kinases peptide substrates
GEEPLYWSFPAKKK